European Patent Application EP 4 599 889 A2, published August 13, 2025. Title: siRNA and their use in methods and compositions for inhibiting the expression of the NRARP gene. Applicant: Sylentis SAU. The sequence listing filed with the application follows.

SEQUENCE LISTING (66 sequences)

SEQ ID NO: 1 - DNA, 19 bp, synthetic construct
  misc_feature 1..19: note = cDNA
  source 1..19: mol_type = other DNA
caccaggacatcgtgctct

SEQ ID NO: 2 - DNA, 19 bp, synthetic construct
  misc_feature 1..19: note = cDNA
  source 1..19: mol_type = other DNA
acatcgtgctctatctcat

SEQ ID NO: 3 - DNA, 19 bp, synthetic construct
  misc_feature 1..19: note = cDNA
  source 1..19: mol_type = other DNA
aggacatcgtgctctatct

SEQ ID NO: 4 - DNA, 19 bp, synthetic construct
  misc_feature 1..19: note = cDNA
  source 1..19: mol_type = other DNA
gacatcgtgctctatctca

SEQ ID NO: 5 - DNA, 19 bp, synthetic construct
  misc_feature 1..19: note = cDNA
  source 1..19: mol_type = other DNA
tgctctatctcatcaccaa

SEQ ID NO: 6 - DNA, 19 bp, synthetic construct
  misc_feature 1..19: note = cDNA
  source 1..19: mol_type = other DNA
ccaggacatcgtgctctat

SEQ ID NO: 7 - DNA, 19 bp, synthetic construct
  misc_feature 1..19: note = cDNA
  source 1..19: mol_type = other DNA
atcgtgctctatctcatca

SEQ ID NO: 8 - DNA, 19 bp, synthetic construct
  misc_feature 1..19: note = cDNA
  source 1..19: mol_type = other DNA
gtgctctatctcatcacca

SEQ ID NO: 9 - DNA, 19 bp, synthetic construct
  misc_feature 1..19: note = cDNA
  source 1..19: mol_type = other DNA
accaggacatcgtgctcta

SEQ ID NO: 10 - RNA, 19 nt, synthetic construct
  misc_feature 1..19: note = siRNA sense strand
  source 1..19: mol_type = other RNA
caccaggacatcgtgctct

SEQ ID NO: 11 - RNA, 19 nt, synthetic construct
  misc_feature 1..19: note = siRNA sense strand
  source 1..19: mol_type = other RNA
acatcgtgctctatctcat

SEQ ID NO: 12 - RNA, 19 nt, synthetic construct
  misc_feature 1..19: note = siRNA sense strand
  source 1..19: mol_type = other RNA
aggacatcgtgctctatct

SEQ ID NO: 13 - RNA, 19 nt, synthetic construct
  misc_feature 1..19: note = siRNA
  source 1..19: mol_type = other RNA
gacatcgtgctctatctca

SEQ ID NO: 14 - RNA, 19 nt, synthetic construct
  misc_feature 1..19: note = siRNA
  source 1..19: mol_type = other RNA
tgctctatctcatcaccaa

SEQ ID NO: 15 - RNA, 19 nt, synthetic construct
  misc_feature 1..19: note = siRNA
  source 1..19: mol_type = other RNA
ccaggacatcgtgctctat

SEQ ID NO: 16 - RNA, 19 nt, synthetic construct
  misc_feature 1..19: note = siRNA
  source 1..19: mol_type = other RNA
atcgtgctctatctcatca

SEQ ID NO: 17 - RNA, 19 nt, synthetic construct
  misc_feature 1..19: note = siRNA
  source 1..19: mol_type = other RNA
gtgctctatctcatcacca

SEQ ID NO: 18 - RNA, 19 nt, synthetic construct
  misc_feature 1..19: note = siRNA
  source 1..19: mol_type = other RNA
accaggacatcgtgctcta

SEQ ID NO: 19 - RNA, 22 nt, synthetic construct
  misc_feature 1..22: note = siRNA
  modified_base 1: mod_base = cm
  misc_feature 4: note = phosphothioate bond
  modified_base 13: mod_base = um
  source 1..22: mol_type = other RNA
  modified_base 3: mod_base = cm
  modified_base 5: mod_base = cm
  modified_base 11: mod_base = cm
  modified_base 14: mod_base = cm
  modified_base 16: mod_base = um
  modified_base 19: mod_base = um
  modified_base 22: mod_base = um
  misc_feature 7: note = phosphothioate bond
  misc_feature 20: note = phosphothioate bond
nannnanggananngngcnncn

SEQ ID NO: 20 - RNA, 20 nt, synthetic construct
  misc_feature 1..20: note = siRNA
  misc_feature 2: note = phosphothioate bond
  modified_base 16: mod_base = um
  modified_base 18: mod_base = gm
  source 1..20: mol_type = other RNA
  modified_base 20: mod_base = gm
  modified_base 19: mod_base = um
angagcacgatgtccngnnn

SEQ ID NO: 21 - RNA, 22 nt, synthetic construct
  misc_feature 1..22: note = siRNA
  modified_base 1: mod_base = cm
  misc_feature 4: note = phosphothioate bond
  modified_base 13: mod_base = um
  source 1..22: mol_type = other RNA
  misc_feature 7: note = phosphothioate bond
  misc_feature 20: note = phosphothioate bond
  modified_base 3: mod_base = cm
  modified_base 5: mod_base = cm
  modified_base 11: mod_base = cm
  modified_base 14: mod_base = cm
  modified_base 16: mod_base = um
  modified_base 19: mod_base = um
  modified_base 22: mod_base = um
nannnanggananngngcnncn

SEQ ID NO: 22 - RNA, 20 nt, synthetic construct
  misc_feature 1..20: note = siRNA
  misc_feature 2: note = phosphothioate bond
  modified_base 16: mod_base = OTHER; note = uridine with 4'-thioribose modification
  modified_base 17: mod_base = gm
  source 1..20: mol_type = other RNA
  modified_base 19: mod_base = OTHER; note = uridine with 4'-thioribose modification
  modified_base 20: mod_base = gm
angagcacgatgtccnngnn

SEQ ID NO: 23 - RNA, 22 nt, synthetic construct
  misc_feature 1..22: note = siRNA
  modified_base 1: mod_base = cm
  misc_feature 4: note = phosphothioate bond
  modified_base 13: mod_base = um
  source 1..22: mol_type = other RNA
  misc_feature 7: note = phosphothioate bond
  misc_feature 20: note = phosphothioate bond
  modified_base 16: mod_base = um
  modified_base 19: mod_base = um
  modified_base 22: mod_base = um
  modified_base 3: mod_base = cm
  modified_base 5: mod_base = cm
  modified_base 11: mod_base = cm
  modified_base 14: mod_base = cm
nannnanggananngngcnncn

SEQ ID NO: 24 - RNA, 20 nt, synthetic construct
  misc_feature 1..20: note = siRNA
  modified_base 16: mod_base = OTHER; note = 5pU (5-Propynyluracile 3')
  source 1..20: mol_type = other RNA
  misc_feature 2: note = phosphothioate bond
  modified_base 19: mod_base = OTHER; note = 5pU (5-Propynyluracile 3')
angagcacgatgtccnggng

SEQ ID NO: 25 - RNA, 22 nt, synthetic construct
  misc_feature 1..22: note = siRNA
  modified_base 1: mod_base = cm
  misc_feature 4: note = phosphothioate bond
  modified_base 13: mod_base = um
  source 1..22: mol_type = other RNA
  misc_feature 7: note = phosphothioate bond
  misc_feature 20: note = phosphothioate bond
  modified_base 16: mod_base = um
  modified_base 19: mod_base = um
  modified_base 22: mod_base = um
  modified_base 3: mod_base = cm
  modified_base 5: mod_base = cm
  modified_base 11: mod_base = cm
  modified_base 14: mod_base = cm
nannnanggananngngcnncn

SEQ ID NO: 26 - RNA, 19 nt, synthetic construct
  misc_feature 1..19: note = siRNA
  modified_base 15: mod_base = m5u
  modified_base 19: mod_base = OTHER; note = 2'F Guanosine
  source 1..19: mol_type = other RNA
  modified_base 18: mod_base = m5u
agagcacgatgtccnggnn

SEQ ID NO: 27 - RNA, 22 nt, synthetic construct
  misc_feature 1..22: note = siRNA
  modified_base 1: mod_base = cm
  misc_feature 4: note = phosphothioate bond
  modified_base 13: mod_base = um
  source 1..22: mol_type = other RNA
  misc_feature 7: note = phosphothioate bond
  misc_feature 20: note = phosphothioate bond
  modified_base 3: mod_base = cm
  modified_base 5: mod_base = cm
  modified_base 11: mod_base = cm
  modified_base 14: mod_base = cm
  modified_base 16: mod_base = um
  modified_base 19: mod_base = um
  modified_base 22: mod_base = um
nannnanggananngngcnncn

SEQ ID NO: 28 - RNA, 19 nt, synthetic construct
  misc_feature 1..19: note = siRNA
  modified_base 15: mod_base = um
  modified_base 17: mod_base = gm
  modified_base 19: mod_base = OTHER; note = 2'F Guanosine
  source 1..19: mol_type = other RNA
  modified_base 18: mod_base = um
agagcacgatgtccngnnn

SEQ ID NO: 29 - RNA, 22 nt, synthetic construct
  misc_feature 1..22: note = siRNA
  modified_base 1: mod_base = OTHER; note = 2'F cytidine
  modified_base 3: mod_base = cm
  misc_feature 4: note = phosphothioate bond
  modified_base 13: mod_base = um
  source 1..22: mol_type = other RNA
  misc_feature 7: note = phosphothioate bond
  misc_feature 20: note = phosphothioate bond
  modified_base 5: mod_base = cm
  modified_base 11: mod_base = cm
  modified_base 14: mod_base = cm
  modified_base 16: mod_base = um
  modified_base 19: mod_base = um
  modified_base 22: mod_base = um
nannnanggananngngcnncn

SEQ ID NO: 30 - RNA, 19 nt, synthetic construct
  misc_feature 1..19: note = siRNA
  modified_base 15: mod_base = um
  modified_base 17: mod_base = gm
  modified_base 19: mod_base = OTHER; note = 2'F Guanosine
  source 1..19: mol_type = other RNA
  modified_base 18: mod_base = um
agagcacgatgtccngnnn

SEQ ID NO: 31 - skipped

SEQ ID NO: 32 - RNA, 19 nt, synthetic construct
  misc_feature 1..19: note = siRNA
  modified_base 1: mod_base = OTHER; note = 2'F Adenosine
  modified_base 5: mod_base = cm
  modified_base 6: mod_base = OTHER; note = 2'-o-methyladenosine
  modified_base 10: mod_base = um
  source 1..19: mol_type = other RNA
  modified_base 15: mod_base = um
  modified_base 18: mod_base = um
ngagnncgangtccnggng

SEQ ID NO: 33 - skipped

SEQ ID NO: 34 - RNA, 19 nt, synthetic construct
  misc_feature 1..19: note = siRNA
  modified_base 1: mod_base = OTHER; note = 2'-o-methyladenosine
  modified_base 5: mod_base = cm
  modified_base 10: mod_base = um
  source 1..19: mol_type = other RNA
  modified_base 6: mod_base = OTHER; note = 2'-o-methyladenosine
  modified_base 15: mod_base = um
  modified_base 18: mod_base = um
ngagnncgangtccnggng

SEQ ID NO: 35 - RNA, 21 nt, synthetic construct
  misc_feature 1..21: note = siRNA
  modified_base 20: mod_base = OTHER; note = deoxithymine (2'H thymine)
  source 1..21: mol_type = other RNA
  modified_base 21: mod_base = OTHER; note = deoxithymine (2'H thymine)
caccaggacatcgtgctctnn

SEQ ID NO: 36 - RNA, 21 nt, synthetic construct
  misc_feature 1..21: note = siRNA
  modified_base 20: mod_base = OTHER; note = deoxithymine (2'H thymine)
  source 1..21: mol_type = other RNA
  modified_base 21: mod_base = OTHER; note = deoxithymine (2'H thymine)
agagcacgatgtcctggtgnn

SEQ ID NO: 37-39 - skipped (3 entries)

SEQ ID NO: 40 - RNA, 19 nt, synthetic construct
  misc_feature 1..19: note = siRNA
  modified_base 5: mod_base = cm
  source 1..19: mol_type = other RNA
agagnacgatgtcctggtg

SEQ ID NO: 41 - RNA, 22 nt, synthetic construct
  misc_feature 1..22: note = siRNA
  misc_feature 4: note = phosphothioate bond
  modified_base 16: mod_base = um
  source 1..22: mol_type = other RNA
  misc_feature 7: note = phosphothioate bond
  misc_feature 20: note = phosphothioate bond
acantcngtgctctanctcnat

SEQ ID NO: 42 - RNA, 19 nt, synthetic construct
  misc_feature 1..19: note = siRNA
  modified_base 15: mod_base = gm
  modified_base 17: mod_base = um
  source 1..19: mol_type = other RNA
  modified_base 19: mod_base = um
atgagatagagcacnangn

SEQ ID NO: 43 - RNA, 22 nt, synthetic construct
  misc_feature 1..22: note = siRNA
  modified_base 2: mod_base = cm
  misc_feature 4: note = phosphothioate bond
  modified_base 9: mod_base = um
  source 1..22: mol_type = other RNA
  modified_base 19: mod_base = cm
  misc_feature 7: note = phosphothioate bond
  misc_feature 20: note = phosphothioate bond
  modified_base 14: mod_base = um
  modified_base 16: mod_base = um
anantcngngctcnanctnnat

SEQ ID NO: 44 - RNA, 19 nt, synthetic construct
  misc_feature 1..19: note = siRNA
  modified_base 15: mod_base = gm
  modified_base 17: mod_base = um
  source 1..19: mol_type = other RNA
  modified_base 19: mod_base = um
atgagatagagcacnangn

SEQ ID NO: 45 - RNA, 22 nt, synthetic construct
  misc_feature 1..22: note = siRNA
  modified_base 2: mod_base = cm
  misc_feature 4: note = phosphothioate bond
  modified_base 9: mod_base = um
  source 1..22: mol_type = other RNA
  misc_feature 7: note = phosphothioate bond
  misc_feature 20: note = phosphothioate bond
  modified_base 19: mod_base = cm
  modified_base 14: mod_base = um
  modified_base 16: mod_base = cm
anantcngngctcnanctnnat

SEQ ID NO: 46 - RNA, 19 nt, synthetic construct
  misc_feature 1..19: note = siRNA
  modified_base 17: mod_base = OTHER; note = 5pU (5-Propynyluracile 3')
  source 1..19: mol_type = other RNA
  modified_base 19: mod_base = OTHER; note = 5pU (5-Propynyluracile 3')
atgagatagagcacgangn

SEQ ID NO: 47 - RNA, 22 nt, synthetic construct
  misc_feature 1..22: note = siRNA
  modified_base 2: mod_base = cm
  misc_feature 4: note = phosphothioate bond
  modified_base 9: mod_base = um
  source 1..22: mol_type = other RNA
  modified_base 19: mod_base = cm
  misc_feature 7: note = phosphothioate bond
  misc_feature 20: note = phosphothioate bond
  modified_base 14: mod_base = um
  modified_base 16: mod_base = um
anantcngngctcnanctnnat

SEQ ID NO: 48 - RNA, 20 nt, synthetic construct
  misc_feature 1..20: note = siRNA
  misc_feature 2: note = phosphothioate bond
  modified_base 18: mod_base = OTHER; note = uridine with 4'-thioribose modification
  source 1..20: mol_type = other RNA
  modified_base 20: mod_base = OTHER; note = uridine with 4'-thioribose modification
antgagatagagcacgangn

SEQ ID NO: 49 - RNA, 22 nt, synthetic construct
  misc_feature 1..22: note = siRNA
  modified_base 2: mod_base = cm
  misc_feature 4: note = phosphothioate bond
  modified_base 9: mod_base = um
  source 1..22: mol_type = other RNA
  modified_base 19: mod_base = cm
  misc_feature 7: note = phosphothioate bond
  misc_feature 20: note = phosphothioate bond
  modified_base 14: mod_base = um
  modified_base 16: mod_base = um
anantcngngctcnanctnnat

SEQ ID NO: 50 - RNA, 19 nt, synthetic construct
  misc_feature 1..19: note = siRNA
  modified_base 17: mod_base = OTHER; note = uridine with 4'-thioribose modification
  modified_base 18: mod_base = gm
  source 1..19: mol_type = other RNA
  modified_base 19: mod_base = OTHER; note = uridine with 4'-thioribose modification
atgagatagagcacgannn

SEQ ID NO: 51 - RNA, 22 nt, synthetic construct
  misc_feature 1..22: note = siRNA
  modified_base 2: mod_base = cm
  misc_feature 4: note = phosphothioate bond
  modified_base 9: mod_base = um
  source 1..22: mol_type = other RNA
  modified_base 19: mod_base = cm
  misc_feature 7: note = phosphothioate bond
  misc_feature 20: note = phosphothioate bond
  modified_base 14: mod_base = um
  modified_base 16: mod_base = um
anantcngngctcnanctnnat

SEQ ID NO: 52 - RNA, 19 nt, synthetic construct
  misc_feature 1..19: note = siRNA
  modified_base 2: mod_base = OTHER; note = uridine with 4'-thioribose modification
  modified_base 18: mod_base = gm
  source 1..19: mol_type = other RNA
  modified_base 17: mod_base = OTHER; note = uridine with 4'-thioribose modification
  modified_base 19: mod_base = OTHER; note = uridine with 4'-thioribose modification
angagatagagcacgannn

SEQ ID NO: 53 - RNA, 22 nt, synthetic construct
  misc_feature 1..22: note = siRNA
  modified_base 2: mod_base = cm
  misc_feature 4: note = phosphothioate bond
  modified_base 9: mod_base = um
  source 1..22: mol_type = other RNA
  misc_feature 7: note = phosphothioate bond
  misc_feature 20: note = phosphothioate bond
  modified_base 19: mod_base = cm
  modified_base 14: mod_base = um
  modified_base 19: mod_base = um
anantcngngctcnanctnnat

SEQ ID NO: 54 - RNA, 20 nt, synthetic construct
  misc_feature 1..20: note = siRNA
  misc_feature 2: note = phosphothioate bond
  modified_base 18: mod_base = OTHER; note = 5pU (5-Propynyluracile 3')
  source 1..20: mol_type = other RNA
  modified_base 20: mod_base = OTHER; note = 5pU (5-Propynyluracile 3')
antgagatagagcacgangn

SEQ ID NO: 55 - skipped

SEQ ID NO: 56 - RNA, 20 nt, synthetic construct
  misc_feature 1..20: note = siRNA
  misc_feature 2: note = phosphothiate bond
  modified_base 18: mod_base = OTHER; note = 5'methyluridine (5mU)
  source 1..20: mol_type = other RNA
  modified_base 20: mod_base = OTHER; note = 5'methyluridine (5mU)
antgagatagagcacgangn

SEQ ID NO: 57 - skipped

SEQ ID NO: 58 - RNA, 19 nt, synthetic construct
  misc_feature 1..19: note = siRNA
  modified_base 2: mod_base = um
  source 1..19: mol_type = other RNA
  modified_base 7: mod_base = um
  modified_base 17: mod_base = um
  modified_base 19: mod_base = um
angaganagagcacgangn

SEQ ID NO: 59 - skipped

SEQ ID NO: 60 - RNA, 19 nt, synthetic construct
  misc_feature 1..19: note = siRNA
  modified_base 1: mod_base = OTHER; note = 2'F Adenosine
  modified_base 2: mod_base = um
  source 1..19: mol_type = other RNA
  modified_base 7: mod_base = um
  modified_base 17: mod_base = um
  modified_base 19: mod_base = um
nngaganagagcacgangn

SEQ ID NO: 61 - RNA, 21 nt, synthetic construct
  misc_feature 1..21: note = siRNA
  modified_base 20: mod_base = OTHER; note = deoxithymine (2'H thymine)
  source 1..21: mol_type = other RNA
  modified_base 21: mod_base = OTHER; note = deoxithymine (2'H thymine)
acatcgtgctctatctcatnn

SEQ ID NO: 62 - RNA, 21 nt, synthetic construct
  misc_feature 1..21: note = siRNA
  modified_base 20: mod_base = OTHER; note = deoxithymine (2'H thymine)
  source 1..21: mol_type = other RNA
  modified_base 21: mod_base = OTHER; note = deoxithymine (2'H thymine)
atgagatagagcacgatgtnn

SEQ ID NO: 63 - skipped

SEQ ID NO: 64 - RNA, 19 nt, synthetic construct
  misc_feature 1..19: note = siRNA
  modified_base 7: mod_base = um
  modified_base 12: mod_base = cm
  source 1..19: mol_type = other RNA
atgaganagagnacgatgt

SEQ ID NO: 65-66 - skipped (2 entries)